European Patent Application EP 4 219 548 A1, published August 2, 2023. Title: SARS-CoV-2 neutralizing antibody or fragment thereof. Applicant: Keio University JAPAN as represented by DIRECTOR GENERAL of National Institute of Infectious Diseases. The sequence listing filed with the application follows.

SEQUENCE LISTING (391 sequences)

SEQ ID NO: 1 - protein, 5 aa, Homo sapiens
NHAIN

SEQ ID NO: 2 - protein, 17 aa, Homo sapiens
WINTNTGNPTYAPGFTG

SEQ ID NO: 3 - protein, 19 aa, Homo sapiens
IPIRDYDYDGSGYYYFLDY

SEQ ID NO: 4 - protein, 11 aa, Homo sapiens
QGDSLRSSSAS

SEQ ID NO: 5 - protein, 7 aa, Homo sapiens
GKTNRPS

SEQ ID NO: 6 - protein, 12 aa, Homo sapiens
NSRDNSGNHPVV

SEQ ID NO: 7 - protein, 5 aa, Homo sapiens
DYAMH

SEQ ID NO: 8 - protein, 17 aa, Homo sapiens
GISRNSAAIAYADSVKG

SEQ ID NO: 9 - protein, 15 aa, Homo sapiens
SPRYGWGSPDYSFDF

SEQ ID NO: 10 - protein, 11 aa, Homo sapiens
RASQNIGTYLN

SEQ ID NO: 11 - protein, 7 aa, Homo sapiens
AASSLQS

SEQ ID NO: 12 - protein, 9 aa, Homo sapiens
QQSFTTPLT

SEQ ID NO: 13 - protein, 5 aa, Homo sapiens
NYWIA

SEQ ID NO: 14 - protein, 17 aa, Homo sapiens
IIHPGDSDIRYRPSLQG

SEQ ID NO: 15 - protein, 13 aa, Homo sapiens
ITTDADSSGLFHY

SEQ ID NO: 16 - protein, 11 aa, Homo sapiens
RASQNIYTWLA

SEQ ID NO: 17 - protein, 7 aa, Homo sapiens
KASSLES

SEQ ID NO: 18 - protein, 8 aa, Homo sapiens
QQYKSAWS

SEQ ID NO: 19 - protein, 5 aa, Homo sapiens
SYDII

SEQ ID NO: 20 - protein, 17 aa, Homo sapiens
WMDPSRGTTGYAQTFQG

SEQ ID NO: 21 - protein, 11 aa, Homo sapiens
HIVVLDRWFDP

SEQ ID NO: 22 - protein, 11 aa, Homo sapiens
QASQDIGNFLN

SEQ ID NO: 23 - protein, 7 aa, Homo sapiens
GASNLET

SEQ ID NO: 24 - protein, 11 aa, Homo sapiens
QHYDNFPPRFT

SEQ ID NO: 25 - protein, 5 aa, Homo sapiens
SYAIS

SEQ ID NO: 26 - protein, 17 aa, Homo sapiens
RIILIFGVANYAQKFQG

SEQ ID NO: 27 - protein, 14 aa, Homo sapiens
GGFYYDSSGYHLDY

SEQ ID NO: 28 - protein, 12 aa, Homo sapiens
RPSQSVSSSYLA

SEQ ID NO: 29 - protein, 7 aa, Homo sapiens
GASSRAT

SEQ ID NO: 30 - protein, 9 aa, Homo sapiens
HQYGSSPRT

SEQ ID NO: 31 - protein, 5 aa, Homo sapiens
HYPMH

SEQ ID NO: 32 - protein, 17 aa, Homo sapiens
VISYDGSNQHYVDSVKG

SEQ ID NO: 33 - protein, 11 aa, Homo sapiens
LITMIRGVPDY

SEQ ID NO: 34 - protein, 11 aa, Homo sapiens
RASQSISNYLN

SEQ ID NO: 35 - protein, 7 aa, Homo sapiens
AASSLQS

SEQ ID NO: 36 - protein, 9 aa, Homo sapiens
LQTYSTPRT

SEQ ID NO: 37 - protein, 5 aa, Homo sapiens
GYYMH

SEQ ID NO: 38 - protein, 17 aa, Homo sapiens
WINPNSGASNYTRKFQG

SEQ ID NO: 39 - protein, 13 aa, Homo sapiens
DLAFSMVRGALDY

SEQ ID NO: 40 - protein, 14 aa, Homo sapiens
TGTSSDVGGYNYVS

SEQ ID NO: 41 - protein, 7 aa, Homo sapiens
EVSKRPS

SEQ ID NO: 42 - protein, 10 aa, Homo sapiens
NSYAGNNNWV

SEQ ID NO: 43 - protein, 5 aa, Homo sapiens
NSAVQ

SEQ ID NO: 44 - protein, 17 aa, Homo sapiens
WIVVGSGNPNYAQKFQE

SEQ ID NO: 45 - protein, 12 aa, Homo sapiens
FPYYYDNSGSGP

SEQ ID NO: 46 - protein, 11 aa, Homo sapiens
QASQDIRNNLN

SEQ ID NO: 47 - protein, 7 aa, Homo sapiens
DASNLET

SEQ ID NO: 48 - protein, 10 aa, Homo sapiens
QQYANLPPFT

SEQ ID NO: 49 - protein, 5 aa, Homo sapiens
SHYMN

SEQ ID NO: 50 - protein, 16 aa, Homo sapiens
VIYSSGSTYYADSVKG

SEQ ID NO: 51 - protein, 13 aa, Homo sapiens
PNYGGNSIWYFDL

SEQ ID NO: 52 - protein, 11 aa, Homo sapiens
RASQGIGSWLA

SEQ ID NO: 53 - protein, 7 aa, Homo sapiens
AASSLQS

SEQ ID NO: 54 - protein, 9 aa, Homo sapiens
QQANSFPLT

SEQ ID NO: 55 - protein, 5 aa, Homo sapiens
SYYWT

SEQ ID NO: 56 - protein, 16 aa, Homo sapiens
YISYSGSTNYNPSLRS

SEQ ID NO: 57 - protein, 18 aa, Homo sapiens
DYYYDNSGYPDSYYGMDV

SEQ ID NO: 58 - protein, 11 aa, Homo sapiens
RASQRISSWLA

SEQ ID NO: 59 - protein, 7 aa, Homo sapiens
KASTLQS

SEQ ID NO: 60 - protein, 9 aa, Homo sapiens
QQYNSFSWT

SEQ ID NO: 61 - protein, 5 aa, Homo sapiens
NSGMH

SEQ ID NO: 62 - protein, 17 aa, Homo sapiens
VIWYDGSKKYYVDSVKG

SEQ ID NO: 63 - protein, 16 aa, Homo sapiens
DGTVAVRGVMNPFFDY

SEQ ID NO: 64 - protein, 11 aa, Homo sapiens
QASQDISNYLN

SEQ ID NO: 65 - protein, 7 aa, Homo sapiens
DASNLET

SEQ ID NO: 66 - protein, 9 aa, Homo sapiens
QQYDNLPYT

SEQ ID NO: 67 - protein, 5 aa, Homo sapiens
NAWMS

SEQ ID NO: 68 - protein, 19 aa, Homo sapiens
RIKSKTDGGTTDYAAPVKG

SEQ ID NO: 69 - protein, 14 aa, Homo sapiens
ADYDILTGTPASPY

SEQ ID NO: 70 - protein, 11 aa, Homo sapiens
RASQSITNYLN

SEQ ID NO: 71 - protein, 7 aa, Homo sapiens
AASSLQG

SEQ ID NO: 72 - protein, 9 aa, Homo sapiens
QQTYSTLWT

SEQ ID NO: 73 - protein, 5 aa, Homo sapiens
SYAIN

SEQ ID NO: 74 - protein, 17 aa, Homo sapiens
RIIPMFGIANYAQKFQG

SEQ ID NO: 75 - protein, 14 aa, Homo sapiens
SQYYYDSSGYYFDY

SEQ ID NO: 76 - protein, 12 aa, Homo sapiens
RASQSVSSSYLA

SEQ ID NO: 77 - protein, 7 aa, Homo sapiens
GASSRAT

SEQ ID NO: 78 - protein, 8 aa, Homo sapiens
QQYGSSRT

SEQ ID NO: 79 - protein, 5 aa, Homo sapiens
NYKMN

SEQ ID NO: 80 - protein, 17 aa, Homo sapiens
YISSGSDAIYYADSVKG

SEQ ID NO: 81 - protein, 12 aa, Homo sapiens
GGGYNYGECMDV

SEQ ID NO: 82 - protein, 17 aa, Homo sapiens
KSSQSVLYSSNNKNYLA

SEQ ID NO: 83 - protein, 7 aa, Homo sapiens
WASTRES

SEQ ID NO: 84 - protein, 9 aa, Homo sapiens
QHYYSPPPT

SEQ ID NO: 85 - protein, 5 aa, Homo sapiens
SNYMT

SEQ ID NO: 86 - protein, 16 aa, Homo sapiens
VLYSGGSTFYADSVKG

SEQ ID NO: 87 - protein, 9 aa, Homo sapiens
DLQELGVDC

SEQ ID NO: 88 - protein, 11 aa, Homo sapiens
RASQGISSYLA

SEQ ID NO: 89 - protein, 7 aa, Homo sapiens
AASTLQS

SEQ ID NO: 90 - protein, 8 aa, Homo sapiens
QQLDSYPR

SEQ ID NO: 91 - protein, 5 aa, Homo sapiens
NRAIH

SEQ ID NO: 92 - protein, 17 aa, Homo sapiens
WINAGKGNTKYSQKFQG

SEQ ID NO: 93 - protein, 10 aa, Homo sapiens
GDGYNYGYDS

SEQ ID NO: 94 - protein, 11 aa, Homo sapiens
GGTNIGSKSVH

SEQ ID NO: 95 - protein, 7 aa, Homo sapiens
DDSDRPS

SEQ ID NO: 96 - protein, 13 aa, Homo sapiens
QVWDSTSDLPEVV

SEQ ID NO: 97 - protein, 5 aa, Homo sapiens
SNYMS

SEQ ID NO: 98 - protein, 16 aa, Homo sapiens
VIYSGGSTYYADSVKG

SEQ ID NO: 99 - protein, 11 aa, Homo sapiens
GELDLPYGMDV

SEQ ID NO: 100 - protein, 13 aa, Homo sapiens
SGSSSNIGNNYVS

SEQ ID NO: 101 - protein, 7 aa, Homo sapiens
DTNKRPS

SEQ ID NO: 102 - protein, 11 aa, Homo sapiens
GTWDRSLSAGV

SEQ ID NO: 103 - protein, 5 aa, Homo sapiens
RNYMT

SEQ ID NO: 104 - protein, 16 aa, Homo sapiens
VIYSGGSTFYADSVKG

SEQ ID NO: 105 - protein, 9 aa, Homo sapiens
DRGEDVFDI

SEQ ID NO: 106 - protein, 11 aa, Homo sapiens
RASQGISSYLA

SEQ ID NO: 107 - protein, 7 aa, Homo sapiens
AASTLQS

SEQ ID NO: 108 - protein, 10 aa, Homo sapiens
QQLNSYPGYT

SEQ ID NO: 109 - protein, 5 aa, Homo sapiens
SNYLA

SEQ ID NO: 110 - protein, 16 aa, Homo sapiens
LIYPGGSTFYADSVKG

SEQ ID NO: 111 - protein, 8 aa, Homo sapiens
LYRRGGDS

SEQ ID NO: 112 - protein, 11 aa, Homo sapiens
QASQDIRNYLN

SEQ ID NO: 113 - protein, 7 aa, Homo sapiens
DASNLQT

SEQ ID NO: 114 - protein, 9 aa, Homo sapiens
QQYDNLPIT

SEQ ID NO: 115 - protein, 5 aa, Homo sapiens
SYSMN

SEQ ID NO: 116 - protein, 17 aa, Homo sapiens
YISGSSSTIYYADSVKG

SEQ ID NO: 117 - protein, 11 aa, Homo sapiens
SEWLLPRFFDY

SEQ ID NO: 118 - protein, 13 aa, Homo sapiens
TGNRNNIGSYPVG

SEQ ID NO: 119 - protein, 6 aa, Homo sapiens
GNSPPS

SEQ ID NO: 120 - protein, 11 aa, Homo sapiens
STWDYSLSAVV

SEQ ID NO: 121 - protein, 5 aa, Homo sapiens
SNYMN

SEQ ID NO: 122 - protein, 16 aa, Homo sapiens
VIYSGGSTFYADSVKG

SEQ ID NO: 123 - protein, 10 aa, Homo sapiens
DLDTQGGMDV

SEQ ID NO: 124 - protein, 12 aa, Homo sapiens
RASQGVSSSYLA

SEQ ID NO: 125 - protein, 7 aa, Homo sapiens
GASTRAT

SEQ ID NO: 126 - protein, 9 aa, Homo sapiens
QLYGSSPGT

SEQ ID NO: 127 - protein, 5 aa, Homo sapiens
SYAMH

SEQ ID NO: 128 - protein, 17 aa, Homo sapiens
VISPDGKNKYYVDSVKG

SEQ ID NO: 129 - protein, 17 aa, Homo sapiens
TQSLWFGQFYYIYGMDV

SEQ ID NO: 130 - protein, 13 aa, Homo sapiens
TGSSGSIASNYVQ

SEQ ID NO: 131 - protein, 7 aa, Homo sapiens
EDTERPS

SEQ ID NO: 132 - protein, 9 aa, Homo sapiens
QSYDSNNVV

SEQ ID NO: 133 - protein, 5 aa, Homo sapiens
DYAIH

SEQ ID NO: 134 - protein, 17 aa, Homo sapiens
LISYDGNNKYYADSVKG

SEQ ID NO: 135 - protein, 12 aa, Homo sapiens
DAEGGWVAALDY

SEQ ID NO: 136 - protein, 14 aa, Homo sapiens
TGTSSDVGGYNYVS

SEQ ID NO: 137 - protein, 7 aa, Homo sapiens
EVSKRPS

SEQ ID NO: 138 - protein, 10 aa, Homo sapiens
CSYAGTYPYV

SEQ ID NO: 139 - protein, 5 aa, Homo sapiens
NYTIS

SEQ ID NO: 140 - protein, 17 aa, Homo sapiens
RIIPIFDIVNYAQKFQG

SEQ ID NO: 141 - protein, 17 aa, Homo sapiens
DGVLYDTSGYLYDAFDI

SEQ ID NO: 142 - protein, 11 aa, Homo sapiens
RASQGINNYLA

SEQ ID NO: 143 - protein, 7 aa, Homo sapiens
AASSLQS

SEQ ID NO: 144 - protein, 9 aa, Homo sapiens
LHYNSYPWT

SEQ ID NO: 145 - protein, 5 aa, Homo sapiens
TYYMH

SEQ ID NO: 146 - protein, 17 aa, Homo sapiens
IINPDGGSISYAQKFQG

SEQ ID NO: 147 - protein, 13 aa, Homo sapiens
GLSPTFSSSWFDN

SEQ ID NO: 148 - protein, 11 aa, Homo sapiens
RASQSVSSNLA

SEQ ID NO: 149 - protein, 7 aa, Homo sapiens
GASTRDT

SEQ ID NO: 150 - protein, 9 aa, Homo sapiens
QQYKNWLLT

SEQ ID NO: 151 - protein, 5 aa, Homo sapiens
DYAMH

SEQ ID NO: 152 - protein, 17 aa, Homo sapiens
GISWNKGNIDYADSVKG

SEQ ID NO: 153 - protein, 16 aa, Homo sapiens
DCHYDSPGYFPNCLHS

SEQ ID NO: 154 - protein, 11 aa, Homo sapiens
RASQGINTYLA

SEQ ID NO: 155 - protein, 7 aa, Homo sapiens
TASTLQS

SEQ ID NO: 156 - protein, 9 aa, Homo sapiens
QQVHSYPLT

SEQ ID NO: 157 - DNA, 385 bp, Homo sapiens
caggtgcagctggtgcaatctgggtctgagttgaagaagcctggggcctcagtgaagatttcctgcaaggcttctggatacaccttcattaaccatgctataaattgggtgcgacaggcccctggacaagggcttgagtggatgggatggatcaacaccaacactgggaacccaacgtatgccccgggcttcacaggacggtttgtcttctccttggacacctctgtcagcacggcatatctgcagatcagcagcctaaaggctgaggacactgccgtgtattactgtgcgagaattcctataagagattatgactatgatggcagtggttattactacttccttgactactggggccagggaaccctggtcaccgtctcctcag

SEQ ID NO: 158 - protein, 128 aa, Homo sapiens
QVQLVQSGSELKKPGASVKISCKASGYTFINHAINWVRQAPGQGLEWMGWINTNTGNPTYAPGFTGRFVFSLDTSVSTAYLQISSLKAEDTAVYYCARIPIRDYDYDGSGYYYFLDYWGQGTLVTVSS

SEQ ID NO: 159 - DNA, 328 bp, Homo sapiens
tcctatgagctgactcaggaccctgctgtgtctgtggccttgggacagacagtcaggatcacatgccaaggagacagcctcagaagctcttctgcgagctggtaccagcagaagccaggacaggcccctgtacttgtcatctacggtaaaaccaaccggccctcagggatcccagaccgattctctggctccagctcaggaaacacagcttccttgaccatcactggggctcaggcggaagatgaggctgactattactgtaattcccgggacaacagtggtaaccatcccgtggtattcggcggagggaccaagctgaccgtcctag

SEQ ID NO: 160 - protein, 109 aa, Homo sapiens
SYELTQDPAVSVALGQTVRITCQGDSLRSSSASWYQQKPGQAPVLVIYGKTNRPSGIPDRFSGSSSGNTASLTITGAQAEDEADYYCNSRDNSGNHPVVFGGGTKLTVL

SEQ ID NO: 161 - DNA, 373 bp, Homo sapiens
gaagtgcagctggtggagtctgggggaggcttggtacagcctggcaggtccctgagagtctcctgtgcagcctctggattcacctttgatgattatgccatgcactgggtccggcaaactccacggaagggcctggagtgggtcgcaggtatcagtagaaatagtgctgccatagcctacgcggactctgtgaagggccgattcaccatctccagagacaacgccaagaactccgtgtttctacaaatgaacggtctgagagctgacgacacggccttgtattattgtgtaaagtcgccgagatatggttgggggagtcccgactattccttcgatttctggggccgtggcaccctggtcactgtctcctcag

SEQ ID NO: 162 - protein, 124 aa, Homo sapiens
EVQLVESGGGLVQPGRSLRVSCAASGFTFDDYAMHWVRQTPRKGLEWVAGISRNSAAIAYADSVKGRFTISRDNAKNSVFLQMNGLRADDTALYYCVKSPRYGWGSPDYSFDFWGRGTLVTVSS

SEQ ID NO: 163 - DNA, 322 bp, Homo sapiens
gacatccagttgacccagtctccatcctccctgtctgcatctgtgggagacagagtcaccatcacttgccgggcaagtcagaacattggcacctatttaaattggtatcagcaggaaccagggaaagcccctaaactcctgatctatgctgcatccagtttgcaaagtggggtcccatcaaggttcagtggcagtggatctgggacagatttcactctcaccatcagcagtctgcaacctgaagattttgcaacttactgctgtcaacagagtttcactacccctctgacgttcggccaggggaccaaggtggaaatcaagc

SEQ ID NO: 164 - protein, 107 aa, Homo sapiens
DIQLTQSPSSLSASVGDRVTITCRASQNIGTYLNWYQQEPGKAPKLLIYAASSLQSGVPSRFSGSGSGTDFTLTISSLQPEDFATYCCQQSFTTPLTFGQGTKVEIK

SEQ ID NO: 165 - DNA, 367 bp, Homo sapiens
caggtccagctggtgcagtctggagcagaggtgaaaaagcccggggagtctctgatgatctcctgtaaggcttctggatacaactttcgcaactactggatcgcctgggtgcgccagatgcccgggaaaggcctggagtggatggggatcatccatcctggtgactctgatatcagatataggccgtccctccaaggccacgtcaccatctcagccgacaagtccatcaccaccgcctacctgcagtggggaagcctgaaggcctcggacaccgccatgtattactgtacgagaataaccaccgacgctgatagtagtggtctctttcactactggggccagggaaccctggtcaccgtctcctcag

SEQ ID NO: 166 - protein, 122 aa, Homo sapiens
QVQLVQSGAEVKKPGESLMISCKASGYNFRNYWIAWVRQMPGKGLEWMGIIHPGDSDIRYRPSLQGHVTISADKSITTAYLQWGSLKASDTAMYYCTRITTDADSSGLFHYWGQGTLVTVSS

SEQ ID NO: 167 - DNA, 319 bp, Homo sapiens
gaaattgtgttgacacagtctccttccaccctgtctgcatctgtgggagacagagtcaccatcacttgccgggccagtcagaatatttatacctggttggcctggtatcagcggaaaccagggaaagcccctaaagtcctgatctataaggcgtctagtttagaaagtggggtcccgtcaaggttcagcggcagtggatctgggacagaattcactctcaccatcagcagtctgcagcctgatgattttgcaacttattactgccaacagtataaaagtgcgtggtcgttcggccaagggaccaaggtggaaatcaaac

SEQ ID NO: 168 - protein, 106 aa, Homo sapiens
EIVLTQSPSTLSASVGDRVTITCRASQNIYTWLAWYQRKPGKAPKVLIYKASSLESGVPSRFSGSGSGTEFTLTISSLQPDDFATYYCQQYKSAWSFGQGTKVEIK

SEQ ID NO: 169 - DNA, 361 bp, Homo sapiens
gaggtgcagctggtgcagtctggggctgaggtgaagaagcctggggcctcagtgaaggtctcctgcaaggcttctggttacaccttcaccagttatgatatcatctgggttcgacaggccactggacaagggcttgagtggatgggatggatggaccctagcaggggtaccacaggctatgcacagacgttccagggcagagtcaccatgaccagggacacctccataagcacagcctacttggagctgaacagcctgacatctgaggacacggccgtgtattattgtgtggcccatattgtagtgttggacaggtggttcgacccctggggccagggaaccctggtcaccgtctcctcag

SEQ ID NO: 170 - protein, 120 aa, Homo sapiens
EVQLVQSGAEVKKPGASVKVSCKASGYTFTSYDIIWVRQATGQGLEWMGWMDPSRGTTGYAQTFQGRVTMTRDTSISTAYLELNSLTSEDTAVYYCVAHIVVLDRWFDPWGQGTLVTVSS

SEQ ID NO: 171 - DNA, 328 bp, Homo sapiens
gacatcgtgatgacccagtctccatcctccctgtctgcatctgtaggagacagagtcaccatcacttgccaggcaagtcaggacattggcaactttttaaattggtgtcagcaaaaaccagggcaagcccctaaggtcctgatctacggtgcatccaatttggaaacaggggtcccatcaaggttcagcggaagtggatctgggacagattttactttcaccatcagcagcctgcagcctgaagacattgcaacatattactgtcaacactatgataatttccctccacggttcacttttggccaggggaccaagctggacatcaagc

SEQ ID NO: 172 - protein, 109 aa, Homo sapiens
DIVMTQSPSSLSASVGDRVTITCQASQDIGNFLNWCQQKPGQAPKVLIYGASNLETGVPSRFSGSGSGTDFTFTISSLQPEDIATYYCQHYDNFPPRFTFGQGTKLDIK

SEQ ID NO: 173 - DNA, 370 bp, Homo sapiens
caggttcagctggtgcagtctggggctgaggtgaagaagcctgggtcctcggtgaaggtctcctgcaaggcttctggagacaccttcagcagctatgctatcagctgggtgcgacaggcccctggacaagggcttgagtggatgggaaggatcattcttatttttggtgtagcaaactacgcacagaaattccagggcagagtcacgattaccgcggacaaatccacgagcacagcctacatggagctgagcagcctgagatctgaggacacggccgtgtattactgtgcgagaggggggttttactatgatagtagtggttatcaccttgactactggggccagggaaccctggtcaccgtctcctcag

SEQ ID NO: 174 - protein, 123 aa, Homo sapiens
QVQLVQSGAEVKKPGSSVKVSCKASGDTFSSYAISWVRQAPGQGLEWMGRIILIFGVANYAQKFQGRVTITADKSTSTAYMELSSLRSEDTAVYYCARGGFYYDSSGYHLDYWGQGTLVTVSS

SEQ ID NO: 175 - DNA, 325 bp, Homo sapiens
gaaattgtgttgacgcagtctccaggcaccctgtctttgtctccaggggaaagagccaccctctcctgcaggcccagtcagagtgttagcagcagctacttagcctggtaccagcagagacctggccaggctcccaggctcctcatctatggtgcatccagcagggccactggcatcccagacaggttcagtggcagtgggtctgggacagacttcactctcaccatcagcagactggagcctgaagattttgcagtgtattactgtcaccagtatggtagctcacctcgaacgttcggccaagggaccaaggtggaaatcaaac

SEQ ID NO: 176 - protein, 108 aa, Homo sapiens
EIVLTQSPGTLSLSPGERATLSCRPSQSVSSSYLAWYQQRPGQAPRLLIYGASSRATGIPDRFSGSGSGTDFTLTISRLEPEDFAVYYCHQYGSSPRTFGQGTKVEIK

SEQ ID NO: 177 - DNA, 361 bp, Homo sapiens
gaagtgcagctggtggagtctgggggaggcgtggtccagcctgggaggtccctgagactctcctgtgcagcctctggattcaccttcagtcactatcctatgcactgggtccgccaggctccaggcagggggctggagtgggtggcagttatatcatatgatggaagtaatcaacactacgtagactccgtgaagggccgattcaccatctccagagacaattccaagaacacgctgtatttgcaaatgaacagcctgagagctgaggacacggctgtgtatttctgtgcgagcctaattactatgattcggggagttcccgactactggggccagggaaccctggtcaccgtctcctcag

SEQ ID NO: 178 - protein, 120 aa, Homo sapiens
EVQLVESGGGVVQPGRSLRLSCAASGFTFSHYPMHWVRQAPGRGLEWVAVISYDGSNQHYVDSVKGRFTISRDNSKNTLYLQMNSLRAEDTAVYFCASLITMIRGVPDYWGQGTLVTVSS

SEQ ID NO: 179 - DNA, 322 bp, Homo sapiens
gacatccagatgacccagtctccatcctccctgtctgcatctgttggagacagagtcaccatcacttgccgggcaagtcagagcattagcaactatttaaattggtatcagcagaaaccagggaaagcccctaacctcctaatctttgctgcatccagtttgcaaagtggggtcccatcaaggttcagtggcagtggatctgggacagaattcactctcaccatcagcagtctgcaacctgaagattttgcagcttactactgtctgcagacttacagtacccctcgtacttttggccaggggaccaggctggagatcaaac

SEQ ID NO: 180 - protein, 107 aa, Homo sapiens
DIQMTQSPSSLSASVGDRVTITCRASQSISNYLNWYQQKPGKAPNLLIFAASSLQSGVPSRFSGSGSGTEFTLTISSLQPEDFAAYYCLQTYSTPRTFGQGTRLEIK

SEQ ID NO: 181 - DNA, 367 bp, Homo sapiens
caggtgcagctggtgcagtctggggctgaggtgaagaagcctggggcctcagtgacggtctcctgcaaggcttctggattcctcttcaccggctactatatgcactgggtgcgacaggcccctggacaagggcttgagtggatgggatggatcaaccctaacagtggtgcctcaaactatacacggaaatttcagggcagggtcaccatgaccagggacacgtccatcagcgctacctacatgaaactgagcaggctgacatctgacgacacggccgtgtattactgtgcgagagatctcgcttttagtatggttcggggagctcttgactactggggccagggaaccctggtcaccgtctcctcag

SEQ ID NO: 182 - protein, 122 aa, Homo sapiens
QVQLVQSGAEVKKPGASVTVSCKASGFLFTGYYMHWVRQAPGQGLEWMGWINPNSGASNYTRKFQGRVTMTRDTSISATYMKLSRLTSDDTAVYYCARDLAFSMVRGALDYWGQGTLVTVSS

SEQ ID NO: 183 - DNA, 331 bp, Homo sapiens
cagcttgtgctgactcagcctccctccgcgtccgggtctcctggacagtcagtcaccatctcctgcactggaaccagcagtgacgttggtggttataactatgtctcctggtaccaacatcacccaggcaaagcccccaaactcatgatttatgaggtcagtaagcggccctcaggggtccctgatcgcttctctggctccaagtctggcaacacggcctccctgaccgtctctgggctccaggctgaagatgaggctgattattactgcaactcatatgcaggcaacaacaattgggtcttcggaactgggaccaaggtcaccgtcctag

SEQ ID NO: 184 - protein, 110 aa, Homo sapiens
QLVLTQPPSASGSPGQSVTISCTGTSSDVGGYNYVSWYQHHPGKAPKLMIYEVSKRPSGVPDRFSGSKSGNTASLTVSGLQAEDEADYYCNSYAGNNNWVFGTGTKVTVL

SEQ ID NO: 185 - DNA, 364 bp, Homo sapiens
gaggtgcagctggtgcagtctgggcctgaggtgaagaagcctgggacctcagtgaaggtctcctgcaaggcttctggattcatctttactaactctgctgtgcagtgggtgcgacaggctcgtggacaacgccttgagtggataggatggatcgtcgttggcagtggtaacccaaactacgcacagaagttccaggaaagagtcaccattaccagggacaggtccacaagcacagcctacatggagctgagcagcctgacatccgaggacacggccgtgtactactgtgcggccttcccctattactatgataatagtggctccgggccgtggggccagggaaccctggtcaccgtctcctcag

SEQ ID NO: 186 - protein, 121 aa, Homo sapiens
EVQLVQSGPEVKKPGTSVKVSCKASGFIFTNSAVQWVRQARGQRLEWIGWIVVGSGNPNYAQKFQERVTITRDRSTSTAYMELSSLTSEDTAVYYCAAFPYYYDNSGSGPWGQGTLVTVSS

SEQ ID NO: 187 - DNA, 325 bp, Homo sapiens
gacatccagttgacccagtctccatcctccctgtctgcatctgtaggagacagagtcaccatcacttgccaggcgagtcaggacattaggaacaatttaaattggtatcagcagataccagggaaagcccctaagctcctgatctacgatgcatccaatttggaaacaggggtcccatcaaggttcagtggaagtgcatctgggacagattttactttcaccatcagcagtctgcagcctgaagatgttgcaacatattactgtcaacagtatgctaatctccctccattcactttcggccctgggaccaaagtggatatcaaac

SEQ ID NO: 188 - protein, 108 aa, Homo sapiens
DIQLTQSPSSLSASVGDRVTITCQASQDIRNNLNWYQQIPGKAPKLLIYDASNLETGVPSRFSGSASGTDFTFTISSLQPEDVATYYCQQYANLPPFTFGPGTKVDIK

SEQ ID NO: 189 - DNA, 364 bp, Homo sapiens
gaagtgcagctggtggagtctggaggaggcttggtccagccgggggggtccctgagactctcctgtgaagcctctgaattcaccctcaatagccactacatgaactgggtccgccaggctccagggaaggggctggagtgggtctcagttatttatagcagtggtagcacatactatgcagactccgtgaagggccgattcaccatctccagacacaattccaaggacacgctgtatcttcaaatgaacagcctgaaacctgaggacacggccgtgtattactgtgcgaggccgaactacggtggtaactccatctggtacttcgatctctggggccgtggcaccctggtcactgtctcctcag

SEQ ID NO: 190 - protein, 121 aa, Homo sapiens
EVQLVESGGGLVQPGGSLRLSCEASEFTLNSHYMNWVRQAPGKGLEWVSVIYSSGSTYYADSVKGRFTISRHNSKDTLYLQMNSLKPEDTAVYYCARPNYGGNSIWYFDLWGRGTLVTVSS

SEQ ID NO: 191 - DNA, 322 bp, Homo sapiens
gacatccagatgacccagtctccatcttctgtgtctgcatctgtaggagacagagtcaccatcacttgtcgggcgagtcagggtattggcagctggttggcctggtatcagcagacaccaggtaaagcccctaagctcctgatctatgctgcatccagtttgcaaagtggggtcccatcaaggttcagcggcagtggatctgggacagatttcactctcactatcagcagcctgcagcctgaagactttgcaacttactattgtcaacaggctaacagtttccccctcactttcggcggagggaccaaggtggagatcaaac

SEQ ID NO: 192 - protein, 107 aa, Homo sapiens
DIQMTQSPSSVSASVGDRVTITCRASQGIGSWLAWYQQTPGKAPKLLIYAASSLQSGVPSRFSGSGSGTDFTLTISSLQPEDFATYYCQQANSFPLTFGGGTKVEIK

SEQ ID NO: 193 - DNA, 379 bp, Homo sapiens
caggtgcagctacagcagtcgggcccaggactggtgaagccttcggagaccctgtccctcacctgcactgtctctggtggctccatcagcagttactactggacctggatccgacaacccccagggaagggactggagtggattgcctatatctcttacagtgggagcactaactacaacccctccctcaggagtcgagtcaccatatcagtagacacgtccaagaaccagttctccctgaagctgagctctgtaaccgctgcggacacggccgtgtattactgtgcgagagactattactatgataatagtggttatcctgattcctactacggtatggacgtctggggccaagggaccacggtcaccgtctcctcag

SEQ ID NO: 194 - protein, 126 aa, Homo sapiens
QVQLQQSGPGLVKPSETLSLTCTVSGGSISSYYWTWIRQPPGKGLEWIAYISYSGSTNYNPSLRSRVTISVDTSKNQFSLKLSSVTAADTAVYYCARDYYYDNSGYPDSYYGMDVWGQGTTVTVSS

SEQ ID NO: 195 - DNA, 322 bp, Homo sapiens
gacatccagttgacccagtctccttccaccctgtctgcatctgtaggagacagagtcaccatcacttgccgggccagtcagcgtattagtagctggttggcctggtatcagcagaaaccagggaaagcccctaagctcctgatctataaggcatctactttacaaagtggggtcccatcaagattcagcggcagtggatccgggacagagttcactctcaccatcagcagcctgcagcctgatgattttgccacttattactgccaacagtataatagtttttcttggacgttcggccaagggaccaaggtggaaatcaaac

SEQ ID NO: 196 - protein, 107 aa, Homo sapiens
DIQLTQSPSTLSASVGDRVTITCRASQRISSWLAWYQQKPGKAPKLLIYKASTLQSGVPSRFSGSGSGTEFTLTISSLQPDDFATYYCQQYNSFSWTFGQGTKVEIK

SEQ ID NO: 197 - DNA, 376 bp, Homo sapiens
gaagtgcagctggtggagtctgggggaggcgtggtccagcctgggacgtccccgagactctcctgtgcagcgtctggattcaccttcagtaactctggcatgcactgggtccgccaggctccaggcaaggggctggagtgggtggcagttatatggtatgatggaagtaaaaaatattatgtagactccgtgaagggccgattcaccatctccagagacaattccaagaacacgctgtatctgcaaatgaacagcctgagagccgaggacacggctgtgtattactgtgcgagagatgggaccgtagcagttcggggagttatgaacccgttttttgactactggggccagggaaccctggtcaccgtctcctcag

SEQ ID NO: 198 - protein, 125 aa, Homo sapiens
EVQLVESGGGVVQPGTSPRLSCAASGFTFSNSGMHWVRQAPGKGLEWVAVIWYDGSKKYYVDSVKGRFTISRDNSKNTLYLQMNSLRAEDTAVYYCARDGTVAVRGVMNPFFDYWGQGTLVTVSS

SEQ ID NO: 199 - DNA, 322 bp, Homo sapiens
gacatccagttgacccagtctccatcctccctgtctgcatctgtaggagacagagtcaccatcacttgccaggcgagtcaggacattagcaactatttaaattggtatcagcagataccagggaaagcccctaagctcctgatctacgatgcatccaatttggaaacaggggtcccatcaaggttcagtggaagtggatctgggacagattttactttcaccatcagcagcctgcagcctgaagatattgcaacatattactgtcaacagtatgataatctcccgtacacttttggccaggggaccaagctggagatcaaac

SEQ ID NO: 200 - protein, 107 aa, Homo sapiens
DIQLTQSPSSLSASVGDRVTITCQASQDISNYLNWYQQIPGKAPKLLIYDASNLETGVPSRFSGSGSGTDFTFTISSLQPEDIATYYCQQYDNLPYTFGQGTKLEIK

SEQ ID NO: 201 - DNA, 376 bp, Homo sapiens
caggtgcagctggtggagtctgggggaggcttggtaaagcctggggggtcccttagactctcctgtgcagcctctggattcactttcaataacgcctggatgagctgggtccgccaggctccagggaaggggctggagtgggttggccgtattaaaagcaaaactgatggtgggacaacagactacgctgcacccgtgaaaggcagattcaccttctcaagagatgattcaaaaaacacgctgtatctgcaaatgagcagcctgaaaaccgaggacacagccctgtattactgtaccacagcggattacgatatcttgactggtacccccgcctccccatactggggccagggaaccctggtcaccgtctcctcag

SEQ ID NO: 202 - protein, 125 aa, Homo sapiens
QVQLVESGGGLVKPGGSLRLSCAASGFTFNNAWMSWVRQAPGKGLEWVGRIKSKTDGGTTDYAAPVKGRFTFSRDDSKNTLYLQMSSLKTEDTALYYCTTADYDILTGTPASPYWGQGTLVTVSS

SEQ ID NO: 203 - DNA, 322 bp, Homo sapiens
gacatccagatgacccagtctccatcctccctgtctgcatctgtaggagacagagtcaccatcacttgccgggcaagtcagagcattaccaactatttaaattggtatcagcagaaaccagggaaagcccctaaattcctgatctatgctgcatccagtttgcaaggtggggtcccatcaaggttccgtggcagtggatctgggacagatttcactctcaccatcagcagtctgcaacctgaagattttgcaacttactactgtcaacagacttacagtaccctctggacgttcggccaagggaccaaggtggaaatcaaac

SEQ ID NO: 204 - protein, 107 aa, Homo sapiens
DIQMTQSPSSLSASVGDRVTITCRASQSITNYLNWYQQKPGKAPKFLIYAASSLQGGVPSRFRGSGSGTDFTLTISSLQPEDFATYYCQQTYSTLWTFGQGTKVEIK

SEQ ID NO: 205 - DNA, 370 bp, Homo sapiens
gaggtgcagctggtgcagtctggggctgaggtgaagaagcctgggtcctcggtgaaggtctcctgcaaggcttctggaggcaccttcagcagctatgctatcaactgggtgcgacaggcccctggacaagggcttgagtggatgggaaggatcatccctatgtttgggatagcaaactacgcacagaagttccagggcagagtcacgattaccgcgaacaaatccacgagcacagcctacatggacctgagcagcctgagatctgaggacacggccgtgtattactgtgcgagaagccagtattactatgatagtagtggatactactttgactactggggccagggaaccctggtcaccgtctcctcag

SEQ ID NO: 206 - protein, 123 aa, Homo sapiens
EVQLVQSGAEVKKPGSSVKVSCKASGGTFSSYAINWVRQAPGQGLEWMGRIIPMFGIANYAQKFQGRVTITANKSTSTAYMDLSSLRSEDTAVYYCARSQYYYDSSGYYFDYWGQGTLVTVSS

SEQ ID NO: 207 - DNA, 322 bp, Homo sapiens
gaaattgtgttgacacagtctccaggcaccctgtctttgtctccaggggaaagagccaccctctcctgcagggccagtcaaagtgttagcagcagttacttagcctggtaccagcagaaacctggccaggctcccaggctcctcatctatggtgcatccagcagggccactggcatcccagacaggttcagtggcagtgggtctgggacagacttcactctcaccatcagcagactggagcctgaagattttgcagtgtactactgtcagcagtatggtagctcacggacgttcggccaagggaccaaggtggaaatcaaac

SEQ ID NO: 208 - protein, 107 aa, Homo sapiens
EIVLTQSPGTLSLSPGERATLSCRASQSVSSSYLAWYQQKPGQAPRLLIYGASSRATGIPDRFSGSGSGTDFTLTISRLEPEDFAVYYCQQYGSSRTFGQGTKVEIK

SEQ ID NO: 209 - DNA, 364 bp, Homo sapiens
gaagtgcagctggtggagtctgggggaggcttggtacagcctggggggtccctgagactctcctgtgcagcctctggattcaccttcattaactataaaatgaactgggtccgccaggctccagggaaggggctggagtgggtttcatacattagtagtggtagtgatgccatttactacgcagactctgtgaagggccgattcaccatctccagagacaatgccaagaactcactgtatctgcaaatgaacagcctgagagacgaggacacggctctgtattactgtgcgagagggggtggatacaactatggcgagtgtatggacgtctggggccaagggaccacggtcaccgtctcctcag

SEQ ID NO: 210 - protein, 121 aa, Homo sapiens
EVQLVESGGGLVQPGGSLRLSCAASGFTFINYKMNWVRQAPGKGLEWVSYISSGSDAIYYADSVKGRFTISRDNAKNSLYLQMNSLRDEDTALYYCARGGGYNYGECMDVWGQGTTVTVSS

SEQ ID NO: 211 - DNA, 340 bp, Homo sapiens
gacatccagatgacccagtctccagactccctggctgtgtctctgggcgagagggccaccatcaactgcaagtccagccagagtgttttatacagctccaacaataagaactacttagcttggtaccagcagaaaccaggacagcctcctaaactgctcatttactgggcatctacccgggaatccggggtccctgaccgattcagtggcagcgggtctgggacagatttcactctcaccatcagcagcctgcaggctgaagatgtggcagtttattactgtcagcattattatagtcctcctcccactttcggcggagggaccaaggtggagatcaaac

SEQ ID NO: 212 - protein, 113 aa, Homo sapiens
DIQMTQSPDSLAVSLGERATINCKSSQSVLYSSNNKNYLAWYQQKPGQPPKLLIYWASTRESGVPDRFSGSGSGTDFTLTISSLQAEDVAVYYCQHYYSPPPTFGGGTKVEIK

SEQ ID NO: 213 - DNA, 352 bp, Homo sapiens
gaggtgcagctggtggagtctgggggaggcttggtccagcctggggggtccctgagactctcctgtgcagcctctggaatcatcgtcagtagcaactacatgacctgggtccgccaggctccagggaagggactggagtgggtctcagttctttatagcggtggtagcacattctacgcagactccgtgaagggcagattcaccatctccagagacaattccaagaacatgctgtatcttcaaatgaacagcctgagagccgaggacacggctgtgtactactgtgcgagagatctgcaggagctgggagttgactgctggggccagggaaccctggtcaccgtctcctcag

SEQ ID NO: 214 - protein, 117 aa, Homo sapiens
EVQLVESGGGLVQPGGSLRLSCAASGIIVSSNYMTWVRQAPGKGLEWVSVLYSGGSTFYADSVKGRFTISRDNSKNMLYLQMNSLRAEDTAVYYCARDLQELGVDCWGQGTLVTVSS

SEQ ID NO: 215 - DNA, 319 bp, Homo sapiens
gacatccagttgacccagtctccatccttcctgtctgcttctgtaggagacagagtcaccatcacttgccgggccagtcagggcattagcagttatttagcctggtatcagcaaaaaccagggaaagcccctaagctcctgatctatgctgcatccactttgcaaagtggggtcccatcaaggttcagcggcagtggatctgggacagaattcactctcacaatcagcagcctgcagcctgaagattttgcaacttattactgtcaacagcttgatagttaccctcgtttcggcggagggaccaaggtggagatcaaac

SEQ ID NO: 216 - protein, 106 aa, Homo sapiens
DIQLTQSPSFLSASVGDRVTITCRASQGISSYLAWYQQKPGKAPKLLIYAASTLQSGVPSRFSGSGSGTEFTLTISSLQPEDFATYYCQQLDSYPRFGGGTKVEIK

SEQ ID NO: 217 - DNA, 358 bp, Homo sapiens
caggtgcagcttgtgcagtctggggctgaggtgaagaagcctggggcctcagtgaaggtttcctgcaaggcttctggatacaccctcactaaccgtgctatacattgggtgcgccaggcccccggacaaaggcttgagtggatgggatggatcaacgctggcaaaggtaacacaaaatattcacagaagtttcagggcagagtcaccattaccagggacacatccgcgagcacagcctacatggagctgagcagcctgaaatctgaagacacggctttttattactgtgcgacaggagatggatacaactatggttacgactcctggggccagggaaccctggtcaccgtctcctcag

SEQ ID NO: 218 - protein, 119 aa, Homo sapiens
QVQLVQSGAEVKKPGASVKVSCKASGYTLTNRAIHWVRQAPGQRLEWMGWINAGKGNTKYSQKFQGRVTITRDTSASTAYMELSSLKSEDTAFYYCATGDGYNYGYDSWGQGTLVTVSS

SEQ ID NO: 219 - DNA, 331 bp, Homo sapiens
aattttatgctgactcagccaccctcggtgtcagtggccccaggaaagacggccaggatttcctgtgggggaaccaacattggaagtaaaagtgtgcactggtaccagcagaagccaggccaggcccctgtgctggtcgtccatgatgatagcgaccggccctcagggatccctgagcgattttctgcttccaactctgggaacacggccaccctgaccatcagcagggtcgaagccggggatgaggccgactattactgtcaggtgtgggatagtactagtgatcttccggaggtggtattcggcggagggaccaagctgaccgtcctag

SEQ ID NO: 220 - protein, 110 aa, Homo sapiens
NFMLTQPPSVSVAPGKTARISCGGTNIGSKSVHWYQQKPGQAPVLVVHDDSDRPSGIPERFSASNSGNTATLTISRVEAGDEADYYCQVWDSTSDLPEVVFGGGTKLTVL

SEQ ID NO: 221 - DNA, 358 bp, Homo sapiens
gaggtgcagctgttggagtctggaggaggcttgatccagcctggggggtccctgagactctcctgtgcagcctctgggttaattgtcagtagcaactacatgagttgggtccgccaggctccagggaaggggctggagtgggtctcagtcatttatagcggtggtagcacatactacgcagactccgtgaagggccgattcatctcctccagagacaattccaagaacacgctgtatcttcaaatgaacagcctgagagccgaggacacggccgtgtattactgtgcgagaggggaactggacctcccctacggaatggacgtctggggccaagggaccacggtcaccgtctcctcag

SEQ ID NO: 222 - protein, 119 aa, Homo sapiens
EVQLLESGGGLIQPGGSLRLSCAASGLIVSSNYMSWVRQAPGKGLEWVSVIYSGGSTYYADSVKGRFISSRDNSKNTLYLQMNSLRAEDTAVYYCARGELDLPYGMDVWGQGTTVTVSS

SEQ ID NO: 223 - DNA, 331 bp, Homo sapiens
caggctgtggtgacgcagccgccctcagtgtctgcggccccaggacagaaggtcaccatctcctgctctggaagcagctccaacattgggaataattatgtatcctggtaccagcagctcccaggaacagcccccaaactcctcatttgtgacactaataagcgaccctcagggattcctgaccgattctctggctccaagtctggcacgtcagccaccctgggcatcaccgggctccagactggggacgaggccgattattactgcggaacatgggatagaagcctgagtgcgggggtgttcggcggagggaccaagctgaccgtcctag

SEQ ID NO: 224 - protein, 110 aa, Homo sapiens
QAVVTQPPSVSAAPGQKVTISCSGSSSNIGNNYVSWYQQLPGTAPKLLICDTNKRPSGIPDRFSGSKSGTSATLGITGLQTGDEADYYCGTWDRSLSAGVFGGGTKLTVL

SEQ ID NO: 225 - DNA, 352 bp, Homo sapiens
gaggtgcagctggtggagtctgggggaggcttggtccagcctggggggtccctgagactctcctgtgcagcctctggagtcatcgtcagtagaaactacatgacctgggtccgccaggctccagggaaggggctggagtgggtctcagttatttatagcggtggtagcacattctacgcagactccgtgaagggccgattcaccatctccagagacaattccaagaacacgctgtatcttcaaatgaacagcctgagagctgaggacacggctgtgtattactgtgcgagagatcggggggaggatgtttttgatatctggggccaagggacaatggtcaccgtctcttcag

SEQ ID NO: 226 - protein, 117 aa, Homo sapiens
EVQLVESGGGLVQPGGSLRLSCAASGVIVSRNYMTWVRQAPGKGLEWVSVIYSGGSTFYADSVKGRFTISRDNSKNTLYLQMNSLRAEDTAVYYCARDRGEDVFDIWGQGTMVTVSS

SEQ ID NO: 227 - DNA, 325 bp, Homo sapiens
gacatccagttgacccagtctccatcctccctgtctgcatctgtaggagacagagtcaccatcacttgccgggccagtcagggcattagcagttatttagcctggtatcagcaaaaaccagggaaagcccctaagctcctgatctatgctgcatccactttgcaaagtggggtcccatcaaggttcagcggcagtggatctgggacagatttcactctcaccatcagcagcctgcagcctgaagattttgcaacttattactgtcaacagcttaatagttaccccgggtacacttttggccaggggaccaagctggagatcaaac

SEQ ID NO: 228 - protein, 108 aa, Homo sapiens
DIQLTQSPSSLSASVGDRVTITCRASQGISSYLAWYQQKPGKAPKLLIYAASTLQSGVPSRFSGSGSGTDFTLTISSLQPEDFATYYCQQLNSYPGYTFGQGTKLEIK

SEQ ID NO: 229 - DNA, 349 bp, Homo sapiens
gaagtgcagctggtggagtctggaggaggcttgatccagccgggggggtccctgagactctcctgtgtagcctctgggttcaccgtcagtagcaactatttggcctgggtccgccaggctccaggtcaggggctggagtgggtctcacttatttatcccggtggtagcacattctacgcagactccgtgaagggccgattcaccatctccagaggcaattccaacaacacactgtatcttcaattgaacagcctgagaaccgaggacacggccgtctattactgtgcgagcctctaccgtcgagggggggacagctggggccagggaaccctggtcaccgtctcctcag

SEQ ID NO: 230 - protein, 116 aa, Homo sapiens
EVQLVESGGGLIQPGGSLRLSCVASGFTVSSNYLAWVRQAPGQGLEWVSLIYPGGSTFYADSVKGRFTISRGNSNNTLYLQLNSLRTEDTAVYYCASLYRRGGDSWGQGTLVTVSS

SEQ ID NO: 231 - DNA, 322 bp, Homo sapiens
gacatccagatgacccagtctccatcctccctgtctgcatctgtaggagacagagtcaccatcacttgccaggcgagtcaggacattaggaactatttaaattggtatcagcagaaaccagggaaagcccctaagctcctgatctacgatgcatccaatttgcaaacaggggtcccatcaaggttcagtggaagaggatctgggacagattttactttcaccatcagcagcctgcaggctgaagatattgcaacatattactgtcaacagtatgataatctcccgatcaccttcggccaagggacacgactggagattaaac

SEQ ID NO: 232 - protein, 107 aa, Homo sapiens
DIQMTQSPSSLSASVGDRVTITCQASQDIRNYLNWYQQKPGKAPKLLIYDASNLQTGVPSRFSGRGSGTDFTFTISSLQAEDIATYYCQQYDNLPITFGQGTRLEIK

SEQ ID NO: 233 - DNA, 361 bp, Homo sapiens
gaggtgcagctggtggagtctgggggaggcttggtacagcctggggggtccctgagactctcctgtgcagcctctggattcactttcagtagctatagcatgaactgggtccgccaggctccagggaaggggctggagtgggtttcatacattagtggtagtagtagtaccatatactacgcagactctgtgaagggccgattcaccatctccagagacaacgccaagaactcactgtacctgcaaatgaacagcctgagagccgaggacacggctgtgtattactgtgtgtcctcggaatggctgctacccagattttttgactactggggccagggaaccctggtcaccgtctcctcag

SEQ ID NO: 234 - protein, 120 aa, Homo sapiens
EVQLVESGGGLVQPGGSLRLSCAASGFTFSSYSMNWVRQAPGKGLEWVSYISGSSSTIYYADSVKGRFTISRDNAKNSLYLQMNSLRAEDTAVYYCVSSEWLLPRFFDYWGQGTLVTVSS

SEQ ID NO: 235 - DNA, 328 bp, Homo sapiens
cagcctgtgctgactcaggaagcctcggtgtcagggaccgtgggacagaaggtcaccctgtcctgtactggaaacaggaacaacattggaagttatcctgtgggctggtaccaacagatttctcacggtgctcccaaaactgtgatgtttggaaattctccgccctcagggatccctgaccgcttctttggctcaaggtctgggaccacagcctccctgactatctcgggcctccagcctgaggacgaggctgattattactgttcaacatgggactacagcctcagtgctgtggtattcggcggagggaccaagctgaccgtcctag

SEQ ID NO: 236 - protein, 109 aa, Homo sapiens
QPVLTQEASVSGTVGQKVTLSCTGNRNNIGSYPVGWYQQISHGAPKTVMFGNSPPSGIPDRFFGSRSGTTASLTISGLQPEDEADYYCSTWDYSLSAVVFGGGTKLTVL

SEQ ID NO: 237 - DNA, 355 bp, Homo sapiens
gaggtgcagctggtggagtctggaggaggcttgatccagcctggggggtccctgagactctcctgtgcagcctctgggttcaccgtcagtagcaactacatgaactgggtccgccaggctccagggaaggggctggagtgggtctcagttatttacagcggtggtagtacattctacgcagactccgtgaagggccgattcaccatctccagagacaattccaagaacacgctgtatcttcaaatgaacagcctgagagtcgaggacacggccgtgtattactgtgcgagagatcttgacacccaagggggtatggacgtctggggccaagggaccacggtcaccgtctcctcag

SEQ ID NO: 238 - protein, 118 aa, Homo sapiens
EVQLVESGGGLIQPGGSLRLSCAASGFTVSSNYMNWVRQAPGKGLEWVSVIYSGGSTFYADSVKGRFTISRDNSKNTLYLQMNSLRVEDTAVYYCARDLDTQGGMDVWGQGTTVTVSS

SEQ ID NO: 239 - DNA, 325 bp, Homo sapiens
gaaattgtgttgacgcagtctccaggctccctgtctttgtctccaggggaaagagccaccctctcctgcagggccagtcagggtgttagcagcagctacttagcctggtaccagcacaaacctggccaggctcccaggctcctcatctttggtgcttccaccagggccactggcatcccagacaggttcagtggcagtgggtctgggacagacttcactctcaccatcagcagactggagcctgaagattttgcggtgtattactgtcagctatatggtagctcacccgggacttttggccaggggaccaagctggagatcaaac

SEQ ID NO: 240 - protein, 108 aa, Homo sapiens
EIVLTQSPGSLSLSPGERATLSCRASQGVSSSYLAWYQHKPGQAPRLLIFGASTRATGIPDRFSGSGSGTDFTLTISRLEPEDFAVYYCQLYGSSPGTFGQGTKLEIK

SEQ ID NO: 241 - DNA, 379 bp, Homo sapiens
caggtgcagctggtggagtctgggggaggcgtagtccagcctgggaagtccctgagactctcctgtgcagcctctggattcaccttcagtagctatgccatgcattgggtccgcctggctccaggcaagggactggagtgggtggcagttatatcacccgatggaaagaataaatattatgtagactccgtgaagggccgatccaccatctccagagacaattccaagaacacgctgtatctgctaatgaacagcctgagagctgaggacacggctgtatattactgtgcgactactcaaagtttatggttcgggcaattttactacatctacggcatggacgtctggggccaagggaccacggtcaccgtctcctcag

SEQ ID NO: 242 - protein, 126 aa, Homo sapiens
QVQLVESGGGVVQPGKSLRLSCAASGFTFSSYAMHWVRLAPGKGLEWVAVISPDGKNKYYVDSVKGRSTISRDNSKNTLYLLMNSLRAEDTAVYYCATTQSLWFGQFYYIYGMDVWGQGTTVTVSS

SEQ ID NO: 243 - DNA, 331 bp, Homo sapiens
cagtctgtgctgactcagccccactctgtgtcggagtctccgggaaagacgataaccatctcctgcaccggcagcagtggcagtattgccagcaactatgtgcagtggtaccagcagcgcccgggcagtgcccccaccactgtgatctatgaggatactgaaagaccctctggggtccctgatcggttctctggctccatcgacagctcctccaactctgcctccctcaccatctctggactgaagactgaggacgaggctgactactactgtcagtcttatgatagcaacaatgtggtcttcggcggagggaccaagctgaccgtcctaa

SEQ ID NO: 244 - protein, 110 aa, Homo sapiens
QSVLTQPHSVSESPGKTITISCTGSSGSIASNYVQWYQQRPGSAPTTVIYEDTERPSGVPDRFSGSIDSSSNSASLTISGLKTEDEADYYCQSYDSNNVVFGGGTKLTVL

SEQ ID NO: 245 - DNA, 364 bp, Homo sapiens
caggtgcagctggtggagtctgggggaggcgtggtccagcctgggaggtccctgagactctcctgtgcagcctctggattcaccttcagtgactatgctatacactgggtccgccaggctccaggcagggggctggagcctgtggcacttatttcatatgatggaaataataaatactacgcagactccgtgaagggccgattcaccatctccagagacaattccaagaatgtgttgtatctgcaaatgaacagcctgagagctgacgacacggctgtgtattactgtgcgagagatgcggagggggggtgggtagcagcccttgactactggggccagggaaccctggtcaccgtctcctcag

SEQ ID NO: 246 - protein, 121 aa, Homo sapiens
QVQLVESGGGVVQPGRSLRLSCAASGFTFSDYAIHWVRQAPGRGLEPVALISYDGNNKYYADSVKGRFTISRDNSKNVLYLQMNSLRADDTAVYYCARDAEGGWVAALDYWGQGTLVTVSS

SEQ ID NO: 247 - DNA, 331 bp, Homo sapiens
cagtctgccctgactcagcctcgctcagtgtccgggtctcctggacagtcagtcaccatctcctgcactggaaccagcagtgatgttggtggttataactatgtctcctggtaccaacaccacccaggcaaagcccccaaagtcatgatttatgaggtcagtaagcggccctcaggggtccctgatcgcttctctggctccaagtctggcaccacggcctccctgaccatctctgggctccaggctgaggatgaggctgattattactgctgctcatatgcaggcacctacccgtatgtcttcggaactgggaccaaggtcaccgtcctag

SEQ ID NO: 248 - protein, 110 aa, Homo sapiens
QSALTQPRSVSGSPGQSVTISCTGTSSDVGGYNYVSWYQHHPGKAPKVMIYEVSKRPSGVPDRFSGSKSGTTASLTISGLQAEDEADYYCCSYAGTYPYVFGTGTKVTVL

SEQ ID NO: 249 - DNA, 379 bp, Homo sapiens
caggtgcagctggtgcagtctggggctgaggtgaagaagcctgggtcctcggtgaaggtctcctgcaagacttctggaggcaccttcaccaactatactatcagctgggtgcgacaggcccctggacaagggcttgagtggatgggaaggatcattcctatctttgatatagtaaactacgcacagaagttccagggcagagtcacgattaccgcggacaaatccacgagcacaacctacatggagctgagcagcctgagatctgaggacacggccgtgtattactgtgcgagagatggggtactctatgatactagtggttatttatacgatgcttttgatatctggggccaagggacaatggtcaccgtctcttcag

SEQ ID NO: 250 - protein, 126 aa, Homo sapiens
QVQLVQSGAEVKKPGSSVKVSCKTSGGTFTNYTISWVRQAPGQGLEWMGRIIPIFDIVNYAQKFQGRVTITADKSTSTTYMELSSLRSEDTAVYYCARDGVLYDTSGYLYDAFDIWGQGTMVTVSS

SEQ ID NO: 251 - DNA, 322 bp, Homo sapiens
gacatccagatgacccagtctccatcctcactgtctgcatctgtaggagacagagtcaccatcacttgtcgggcgagtcagggcattaacaattatttagcctggtttcagcagaaaccagggaaagcccctaagtccctgatctatgctgcatccagtttgcaaagtggggtcccaccaaagttcagcggcagtggatctgggacagatttcactctcaccatcagcagcctgcagcctgaagattttgcaacttattactgcctacactataatagttacccttggacgttcggccaagggaccaaggtggaaatcaaac

SEQ ID NO: 252 - protein, 107 aa, Homo sapiens
DIQMTQSPSSLSASVGDRVTITCRASQGINNYLAWFQQKPGKAPKSLIYAASSLQSGVPPKFSGSGSGTDFTLTISSLQPEDFATYYCLHYNSYPWTFGQGTKVEIK

SEQ ID NO: 253 - DNA, 367 bp, Homo sapiens
gaggtgcagctggtgcagtctggggctgaggtgaagaagcctggggcctcagtgaaggtttcctgccaggcatctggatacaccttcatcacctactatatgcactgggtgcgacaggcccctggacaagggcttgagtggatgggaataatcaaccctgatggtggtagcataagttacgcacagaagttccagggcagagtcaccatgaccagggacacgtccacgagcacagtctacatggaactgagcagcctgagatctgaggacacggccgtgtattattgtgcgagagggctcagcccgacatttagcagcagctggtttgacaactggggcctgggaaccctggtcaccgtctcctcag

SEQ ID NO: 254 - protein, 122 aa, Homo sapiens
EVQLVQSGAEVKKPGASVKVSCQASGYTFITYYMHWVRQAPGQGLEWMGIINPDGGSISYAQKFQGRVTMTRDTSTSTVYMELSSLRSEDTAVYYCARGLSPTFSSSWFDNWGLGTLVTVSS

SEQ ID NO: 255 - DNA, 322 bp, Homo sapiens
gatgttgtgatgactcagtctccagccaccctgtctgtgtctccaggggaaagagccaccctctcctgcagggccagtcagagtgttagcagcaacttagcctggtaccagcagaaacctggccaggctcccaggctcctcatctatggtgcatccaccagggacactggtatcccagccaggttcagtggcagtgggtctgggacagagttcactctcaccatcagcagcctgcagtctgaagattttgcagtttatttctgtcagcagtataaaaactggcttctcactttcggcggagggaccaaggtggagatcaaac

SEQ ID NO: 256 - protein, 107 aa, Homo sapiens
DVVMTQSPATLSVSPGERATLSCRASQSVSSNLAWYQQKPGQAPRLLIYGASTRDTGIPARFSGSGSGTEFTLTISSLQSEDFAVYFCQQYKNWLLTFGGGTKVEIK

SEQ ID NO: 257 - DNA, 376 bp, Homo sapiens
gaagtgcagctggtggagtcggggggaggcttggtacagcctggcaggtccctgagactctcctgtgcagcctctggattcacctttgatgattatgccatgcactgggtccggcaagttccagggaagggcctggagtgggtctcaggtattagttggaacaaaggtaacatagactatgcggactctgtgaagggccgattcaccatctccagagacaacgccaagaactccctgtatctgcaaatgaacagtctgagacctgaggacacgggcttatattactgtgcaaaagattgccactatgatagtcctggttatttccctaactgccttcactcctggggccagggaaccctggtcaccgtctcctcag

SEQ ID NO: 258 - protein, 125 aa, Homo sapiens
EVQLVESGGGLVQPGRSLRLSCAASGFTFDDYAMHWVRQVPGKGLEWVSGISWNKGNIDYADSVKGRFTISRDNAKNSLYLQMNSLRPEDTGLYYCAKDCHYDSPGYFPNCLHSWGQGTLVTVSS

SEQ ID NO: 259 - DNA, 322 bp, Homo sapiens
gaaatagtgatgacgcagtctccatcctccctgtctgcatctgtcggagacagagtcaccatcacttgccgggccagtcagggcattaacacttatttagcctggtatcagcaaaaaccagggaaagcccctaaactcctgatctatactgcatccactttgcaaagtggggtcccatcaaggttcagcggcagtggatctgggacagatttcactctcaccatcagcagcctgcagcctgaagattttgcaacttattactgtcaacaggttcatagttaccctctcactttcggcggagggaccaaggtggagatcaaac

SEQ ID NO: 260 - protein, 107 aa, Homo sapiens
EIVMTQSPSSLSASVGDRVTITCRASQGINTYLAWYQQKPGKAPKLLIYTASTLQSGVPSRFSGSGSGTDFTLTISSLQPEDFATYYCQQVHSYPLTFGGGTKVEIK

SEQ ID NO: 261 - protein, 8 aa, Homo sapiens
GYTFINHA

SEQ ID NO: 262 - protein, 8 aa, Homo sapiens
INTNTGNP

SEQ ID NO: 263 - protein, 21 aa, Homo sapiens
ARIPIRDYDYDGSGYYYFLDY

SEQ ID NO: 264 - protein, 6 aa, Homo sapiens
SLRSSS

SEQ ID NO: 265 - protein, 12 aa, Homo sapiens
NSRDNSGNHPVV

SEQ ID NO: 266 - protein, 8 aa, Homo sapiens
GFTFDDYA

SEQ ID NO: 267 - protein, 8 aa, Homo sapiens
ISRNSAAI

SEQ ID NO: 268 - protein, 17 aa, Homo sapiens
VKSPRYGWGSPDYSFDF

SEQ ID NO: 269 - protein, 6 aa, Homo sapiens
QNIGTY

SEQ ID NO: 270 - protein, 9 aa, Homo sapiens
QQSFTTPLT

SEQ ID NO: 271 - protein, 8 aa, Homo sapiens
GYNFRNYW

SEQ ID NO: 272 - protein, 8 aa, Homo sapiens
IHPGDSDI

SEQ ID NO: 273 - protein, 15 aa, Homo sapiens
TRITTDADSSGLFHY

SEQ ID NO: 274 - protein, 6 aa, Homo sapiens
QNIYTW

SEQ ID NO: 275 - protein, 8 aa, Homo sapiens
QQYKSAWS

SEQ ID NO: 276 - protein, 8 aa, Homo sapiens
GYTFTSYD

SEQ ID NO: 277 - protein, 8 aa, Homo sapiens
MDPSRGTT

SEQ ID NO: 278 - protein, 13 aa, Homo sapiens
VAHIVVLDRWFDP

SEQ ID NO: 279 - protein, 6 aa, Homo sapiens
QDIGNF

SEQ ID NO: 280 - protein, 11 aa, Homo sapiens
QHYDNFPPRFT

SEQ ID NO: 281 - protein, 8 aa, Homo sapiens
GDTFSSYA

SEQ ID NO: 282 - protein, 8 aa, Homo sapiens
IILIFGVA

SEQ ID NO: 283 - protein, 16 aa, Homo sapiens
ARGGFYYDSSGYHLDY

SEQ ID NO: 284 - protein, 7 aa, Homo sapiens
QSVSSSY

SEQ ID NO: 285 - protein, 9 aa, Homo sapiens
HQYGSSPRT

SEQ ID NO: 286 - protein, 8 aa, Homo sapiens
GFTFSHYP

SEQ ID NO: 287 - protein, 8 aa, Homo sapiens
ISYDGSNQ

SEQ ID NO: 288 - protein, 13 aa, Homo sapiens
ASLITMIRGVPDY

SEQ ID NO: 289 - protein, 6 aa, Homo sapiens
QSISNY

SEQ ID NO: 290 - protein, 9 aa, Homo sapiens
LQTYSTPRT

SEQ ID NO: 291 - protein, 8 aa, Homo sapiens
GFLFTGYY

SEQ ID NO: 292 - protein, 8 aa, Homo sapiens
INPNSGAS

SEQ ID NO: 293 - protein, 15 aa, Homo sapiens
ARDLAFSMVRGALDY

SEQ ID NO: 294 - protein, 9 aa, Homo sapiens
SSDVGGYNY

SEQ ID NO: 295 - protein, 10 aa, Homo sapiens
NSYAGNNNWV

SEQ ID NO: 296 - protein, 8 aa, Homo sapiens
GFIFTNSA

SEQ ID NO: 297 - protein, 8 aa, Homo sapiens
IVVGSGNP

SEQ ID NO: 298 - protein, 14 aa, Homo sapiens
AAFPYYYDNSGSGP

SEQ ID NO: 299 - protein, 6 aa, Homo sapiens
QDIRNN

SEQ ID NO: 300 - protein, 10 aa, Homo sapiens
QQYANLPPFT

SEQ ID NO: 301 - protein, 8 aa, Homo sapiens
EFTLNSHY

SEQ ID NO: 302 - protein, 7 aa, Homo sapiens
IYSSGST

SEQ ID NO: 303 - protein, 15 aa, Homo sapiens
ARPNYGGNSIWYFDL

SEQ ID NO: 304 - protein, 6 aa, Homo sapiens
QGIGSW

SEQ ID NO: 305 - protein, 9 aa, Homo sapiens
QQANSFPLT

SEQ ID NO: 306 - protein, 8 aa, Homo sapiens
GGSISSYY

SEQ ID NO: 307 - protein, 7 aa, Homo sapiens
ISYSGST

SEQ ID NO: 308 - protein, 20 aa, Homo sapiens
ARDYYYDNSGYPDSYYGMDV

SEQ ID NO: 309 - protein, 6 aa, Homo sapiens
QRISSW

SEQ ID NO: 310 - protein, 9 aa, Homo sapiens
QQYNSFSWT

SEQ ID NO: 311 - protein, 8 aa, Homo sapiens
GFTFSNSG

SEQ ID NO: 312 - protein, 8 aa, Homo sapiens
IWYDGSKK

SEQ ID NO: 313 - protein, 18 aa, Homo sapiens
ARDGTVAVRGVMNPFFDY

SEQ ID NO: 314 - protein, 6 aa, Homo sapiens
QDISNY

SEQ ID NO: 315 - protein, 9 aa, Homo sapiens
QQYDNLPYT

SEQ ID NO: 316 - protein, 8 aa, Homo sapiens
GFTFNNAW

SEQ ID NO: 317 - protein, 10 aa, Homo sapiens
IKSKTDGGTT

SEQ ID NO: 318 - protein, 16 aa, Homo sapiens
TTADYDILTGTPASPY

SEQ ID NO: 319 - protein, 6 aa, Homo sapiens
QSITNY

SEQ ID NO: 320 - protein, 9 aa, Homo sapiens
QQTYSTLWT

SEQ ID NO: 321 - protein, 8 aa, Homo sapiens
GGTFSSYA

SEQ ID NO: 322 - protein, 8 aa, Homo sapiens
IIPMFGIA

SEQ ID NO: 323 - protein, 16 aa, Homo sapiens
ARSQYYYDSSGYYFDY

SEQ ID NO: 324 - protein, 7 aa, Homo sapiens
QSVSSSY

SEQ ID NO: 325 - protein, 8 aa, Homo sapiens
QQYGSSRT

SEQ ID NO: 326 - protein, 8 aa, Homo sapiens
GFTFINYK

SEQ ID NO: 327 - protein, 8 aa, Homo sapiens
ISSGSDAI

SEQ ID NO: 328 - protein, 14 aa, Homo sapiens
ARGGGYNYGECMDV

SEQ ID NO: 329 - protein, 12 aa, Homo sapiens
QSVLYSSNNKNY

SEQ ID NO: 330 - protein, 9 aa, Homo sapiens
QHYYSPPPT

SEQ ID NO: 331 - protein, 8 aa, Homo sapiens
GIIVSSNY

SEQ ID NO: 332 - protein, 7 aa, Homo sapiens
LYSGGST

SEQ ID NO: 333 - protein, 11 aa, Homo sapiens
ARDLQELGVDC

SEQ ID NO: 334 - protein, 6 aa, Homo sapiens
QGISSY

SEQ ID NO: 335 - protein, 8 aa, Homo sapiens
QQLDSYPR

SEQ ID NO: 336 - protein, 8 aa, Homo sapiens
GYTLTNRA

SEQ ID NO: 337 - protein, 8 aa, Homo sapiens
INAGKGNT

SEQ ID NO: 338 - protein, 12 aa, Homo sapiens
ATGDGYNYGYDS

SEQ ID NO: 339 - protein, 6 aa, Homo sapiens
NIGSKS

SEQ ID NO: 340 - protein, 13 aa, Homo sapiens
QVWDSTSDLPEVV

SEQ ID NO: 341 - protein, 8 aa, Homo sapiens
GLIVSSNY

SEQ ID NO: 342 - protein, 7 aa, Homo sapiens
IYSGGST

SEQ ID NO: 343 - protein, 13 aa, Homo sapiens
ARGELDLPYGMDV

SEQ ID NO: 344 - protein, 8 aa, Homo sapiens
SSNIGNNY

SEQ ID NO: 345 - protein, 11 aa, Homo sapiens
GTWDRSLSAGV

SEQ ID NO: 346 - protein, 8 aa, Homo sapiens
GVIVSRNY

SEQ ID NO: 347 - protein, 7 aa, Homo sapiens
IYSGGST

SEQ ID NO: 348 - protein, 11 aa, Homo sapiens
ARDRGEDVFDI

SEQ ID NO: 349 - protein, 6 aa, Homo sapiens
QGISSY

SEQ ID NO: 350 - protein, 10 aa, Homo sapiens
QQLNSYPGYT

SEQ ID NO: 351 - protein, 8 aa, Homo sapiens
GFTVSSNY

SEQ ID NO: 352 - protein, 7 aa, Homo sapiens
IYPGGST

SEQ ID NO: 353 - protein, 10 aa, Homo sapiens
ASLYRRGGDS

SEQ ID NO: 354 - protein, 6 aa, Homo sapiens
QDIRNY

SEQ ID NO: 355 - protein, 9 aa, Homo sapiens
QQYDNLPIT

SEQ ID NO: 356 - protein, 8 aa, Homo sapiens
GFTFSSYS

SEQ ID NO: 357 - protein, 8 aa, Homo sapiens
ISGSSSTI

SEQ ID NO: 358 - protein, 13 aa, Homo sapiens
VSSEWLLPRFFDY

SEQ ID NO: 359 - protein, 8 aa, Homo sapiens
RNNIGSYP

SEQ ID NO: 360 - protein, 11 aa, Homo sapiens
STWDYSLSAVV

SEQ ID NO: 361 - protein, 8 aa, Homo sapiens
GFTVSSNY

SEQ ID NO: 362 - protein, 7 aa, Homo sapiens
IYSGGST

SEQ ID NO: 363 - protein, 12 aa, Homo sapiens
ARDLDTQGGMDV

SEQ ID NO: 364 - protein, 7 aa, Homo sapiens
QGVSSSY

SEQ ID NO: 365 - protein, 9 aa, Homo sapiens
QLYGSSPGT

SEQ ID NO: 366 - protein, 8 aa, Homo sapiens
GFTFSSYA

SEQ ID NO: 367 - protein, 8 aa, Homo sapiens
ISPDGKNK

SEQ ID NO: 368 - protein, 19 aa, Homo sapiens
ATTQSLWFGQFYYIYGMDV

SEQ ID NO: 369 - protein, 8 aa, Homo sapiens
SGSIASNY

SEQ ID NO: 370 - protein, 9 aa, Homo sapiens
QSYDSNNVV

SEQ ID NO: 371 - protein, 8 aa, Homo sapiens
GFTFSDYA

SEQ ID NO: 372 - protein, 8 aa, Homo sapiens
ISYDGNNK

SEQ ID NO: 373 - protein, 14 aa, Homo sapiens
ARDAEGGWVAALDY

SEQ ID NO: 374 - protein, 9 aa, Homo sapiens
SSDVGGYNY

SEQ ID NO: 375 - protein, 10 aa, Homo sapiens
CSYAGTYPYV

SEQ ID NO: 376 - protein, 8 aa, Homo sapiens
GGTFTNYT

SEQ ID NO: 377 - protein, 8 aa, Homo sapiens
IIPIFDIV

SEQ ID NO: 378 - protein, 19 aa, Homo sapiens
ARDGVLYDTSGYLYDAFDI

SEQ ID NO: 379 - protein, 6 aa, Homo sapiens
QGINNY

SEQ ID NO: 380 - protein, 9 aa, Homo sapiens
LHYNSYPWT

SEQ ID NO: 381 - protein, 8 aa, Homo sapiens
GYTFITYY

SEQ ID NO: 382 - protein, 8 aa, Homo sapiens
INPDGGSI

SEQ ID NO: 383 - protein, 15 aa, Homo sapiens
ARGLSPTFSSSWFDN

SEQ ID NO: 384 - protein, 6 aa, Homo sapiens
QSVSSN

SEQ ID NO: 385 - protein, 9 aa, Homo sapiens
QQYKNWLLT

SEQ ID NO: 386 - protein, 8 aa, Homo sapiens
GFTFDDYA

SEQ ID NO: 387 - protein, 8 aa, Homo sapiens
ISWNKGNI

SEQ ID NO: 388 - protein, 18 aa, Homo sapiens
AKDCHYDSPGYFPNCLHS

SEQ ID NO: 389 - protein, 6 aa, Homo sapiens
QGINTY

SEQ ID NO: 390 - protein, 9 aa, Homo sapiens
QQVHSYPLT

SEQ ID NO: 391 - protein, 329 aa, Homo sapiens
STKGPSVFPLAPSSKSTSGGTAALGCLVKDYFPEPVTVSWNSGALTSGVHTFPAVLQSSGLYSLSSVVTVPSSSLGTQTYICNVNHKPSNTKVDKKVEPKSCDKTHTCPPCPAPELLGGPSVFLFPPKPKDTLMISRTPEVTCVVVDVSHEDPEVKFNWYVDGVEVHNAKTKPREEQYASTYRVVSVLTVLHQDWLNGKEYKCKVSNKALPAPIEKTISKAKGQPREPQVYTLPPSRDELTKNQVSLTCLVKGFYPSDIAVEWESNGQPENNYKTTPPVLDSDGSFFLYSKLTVDKSRWQQGNVFSCSVMHEALHNHYTQKSLSLSPGK